European Patent Specification EP 3 504 329 B1, published June 4, 2025. Title: XANTHAN LYASE VARIANTS AND POLYNUCLEOTIDES ENCODING SAME. Applicant: Novozymes A/S. The sequence listing filed with the application follows.

SEQUENCE LISTING (2 sequences)

SEQ ID NO: 1 - DNA, 3111 bp, Paenibacillus sp.
  CDS (1)..(3111)
  mat_peptide (1)..(3111)
gacgagtttgacacgctaagggaaaagtataaggccatgctgaacggagggacaacctataatctctccgacccggatatagcggcgcgtgttaatgccattacggtgactgcccagggatactgggactccatgcttaaagatccgaaccgtaaccgtctttggaacgatgcaccctttggctcggattcgacttccatcaccacgacctacagacacctttatgatatggcgctagcttatacgacttatggctccagtctgcagggcaatgccgcacttaaagcggatattatcagcggtttggactggatgaatgccaatcaattttataatggctgcagccaatatcaaaactggtggcactggcaaattggcggtcccatggccttgaatgatatcgtggcattaatgtacacggagctaaccgcaacacaaatttccaattacatggcggccatttattacacccaagcgagtgttacgatgacgggggcaaaccggctatgggaaagtcaggttattgccatctccggaatcttgaataaggattccgccagagttgccgctggtcgggatggcatcagcgctttgctgccgtatgtcgccaagggtgacggattttacaacgatggatcattcgttcagcatacttattatgcttacaacggtggttatggttcagagctgttatctggcattgcagacttgatatttattttgaatggctcttcatggcaggtaacggatcctaataaaaacaatgtataccgttggatttatgattcctacgagcctttcatctataaagggaatctgatggacatggtccgcggtagagagatctcaaggcatggattgcaggacgataaggcagccgtgactgtgatggcatcgatcattcgtctgtcacaaaccgctgcttccgccgatgctaccgcatttaagagaatggtgaaatattggctgctgctggatacggataagactttccttaaagcagtatcgattgatctgattattgccgcgaaccaactggtgaacgattccaccgttacctctcgaggggagctagtgaaatataaacaattctccggaatggaccgcgctgtacagcttagacctggcttcggttttgggcttagcatgttttccagccggatcggtaattatgagtcgattaatgcagagaacaacaaaggctggcataccggcgacggcatgacctacctttacaatactgacctgagtcagttcaatgaccatttctgggcaactgtggataattaccgattgccgggtaccacagtgctccagaacacgacgcaaaccgcgaacagccgcagcgacaaaagctgggccggaggaacggatattcttgggcaatatggtgtttccggcatggaactgcataccgtaggtaagagcctgacagccaagaaatcctggttcatgtttgacgatgagatcgtcgcgctgggttcaggtattgccagcaccgatggcatcgcaaccgaaacgattgtagagaatcgaaagctcaatagcagcggcaataatgcattgattgttaacgggacggcgaagccgggctcccttggatggtcggaaacaatgaccggaaccaattatattcatctagccggcagcgtacccggctccgatatcggttattattttcctggtggagcagcagtcaaaggcttgcgtgaagcccggtcgggaagctggagctcgctgaattcctccgcatcctggaaggactcgacattgcatacacgcaactttatgacgctttggttcgatcatggcatgaacccgacaaacggtagttattcttatgtgctgcttccgaataagaccagcagtgcggtggccagctatgctgcaacgcctcagatcagcattctggagaattctagctcggcgcaagcggtgaaggagacgcaattgaatgtcaccggaattaacttttggaacgatgagccaaccacggtgggcctggttacttccaatcggaaagcatccgttatgacaaaagaaacggctagtgatttcgagatatccgtttccgacccgacccaaagtaatgtggggaccatctatattgatgtcaacaaaagtgcaaccggattgatttcgaaggataatgaaataacggtcattcagtactacccaaccatgaagtttaaagtcaatgtaaacaattctggcgggaagtcctataaagtaaagtttagcctgacaggaacacccggcagcaacccgtctccaatcccgataccgaatccttacgaagcggaagctttgccaattaacgctctgacagatactcccgtggtttacaatgatgccaatgccagtggtggcaagaagcttggcttcaataacaatgcagtggatgattatgtggagttcagtctggacgtcacacagcccggcacctacgatgtcaaatcccggattatgaaatcaacgaacagcgggatttatcagctgtctattaatgggaccaacgtagggagcgcgcaggatatgttctggacgacctccgagctgtctaaggagtttactatgggctcatacagcttcagcacacccgggagctatttgttccgattaaaaacaaccggcaagaatgtcagttcttcaggatataagctgatgctggacaattttagtctggtatcaacaggtattgatacaacggtgattgtggacaatgccgatgcagctggtgttacgaaggtgggtacttggaccggaaccaatacgcagaccgatcggtacggcgccgactacattcacgatgggaacacggggaaaggtacgaagagcgttacctttactccaaatgtacctatcagtggaacttatcaggtttacatgatgtgggctgcccatacgaatagggcaacgaatgttcccgtagacgtaacgcattcaggcggtacagcaacgctaaatgttaaccaacaaggtaatggtggtgtgtggaatttactgggtacgtatagctttaatgctgggtccacgggggctatcaagatccgtacggacgcgacgaatggatatgttgtagccgatgccgtgaagctggtaaaggtccca

SEQ ID NO: 2 - protein, 1037 aa, Paenibacillus sp.
DEFDTLREKYKAMLNGGTTYNLSDPDIAARVNAITVTAQGYWDSMLKDPNRNRLWNDAPFGSDSTSITTTYRHLYDMALAYTTYGSSLQGNAALKADIISGLDWMNANQFYNGCSQYQNWWHWQIGGPMALNDIVALMYTELTATQISNYMAAIYYTQASVTMTGANRLWESQVIAISGILNKDSARVAAGRDGISALLPYVAKGDGFYNDGSFVQHTYYAYNGGYGSELLSGIADLIFILNGSSWQVTDPNKNNVYRWIYDSYEPFIYKGNLMDMVRGREISRHGLQDDKAAVTVMASIIRLSQTAASADATAFKRMVKYWLLLDTDKTFLKAVSIDLIIAANQLVNDSTVTSRGELVKYKQFSGMDRAVQLRPGFGFGLSMFSSRIGNYESINAENNKGWHTGDGMTYLYNTDLSQFNDHFWATVDNYRLPGTTVLQNTTQTANSRSDKSWAGGTDILGQYGVSGMELHTVGKSLTAKKSWFMFDDEIVALGSGIASTDGIATETIVENRKLNSSGNNALIVNGTAKPGSLGWSETMTGTNYIHLAGSVPGSDIGYYFPGGAAVKGLREARSGSWSSLNSSASWKDSTLHTRNFMTLWFDHGMNPTNGSYSYVLLPNKTSSAVASYAATPQISILENSSSAQAVKETQLNVTGINFWNDEPTTVGLVTSNRKASVMTKETASDFEISVSDPTQSNVGTIYIDVNKSATGLISKDNEITVIQYYPTMKFKVNVNNSGGKSYKVKFSLTGTPGSNPSPIPIPNPYEAEALPINALTDTPVVYNDANASGGKKLGFNNNAVDDYVEFSLDVTQPGTYDVKSRIMKSTNSGIYQLSINGTNVGSAQDMFWTTSELSKEFTMGSYSFSTPGSYLFRLKTTGKNVSSSGYKLMLDNFSLVSTGIDTTVIVDNADAAGVTKVGTWTGTNTQTDRYGADYIHDGNTGKGTKSVTFTPNVPISGTYQVYMMWAAHTNRATNVPVDVTHSGGTATLNVNQQGNGGVWNLLGTYSFNAGSTGAIKIRTDATNGYVVADAVKLVKVP